European Patent Application EP 4 389 914 A1, published June 26, 2024. Title: CRISPR-Cas based method for the detection of non-nucleic acid targets. Applicant: CSEM Centre Suisse d'Electronique et de Microtechnique SA. Application EP. The sequence listing filed with the application follows.

SEQUENCE LISTING (33 sequences)

SEQ ID NO: 1 - DNA, 59 bp, synthetic construct
  source 1..59: mol_type = other DNA
tcttaccctatcagatttagccatgtgtagaccaaattggtctacacatgactaaatct

SEQ ID NO: 2 - DNA, 58 bp, synthetic construct
  source 1..58: mol_type = other DNA
tcttaccctatcagatttagccatgtgtagaccaaatggtctacacatgactaaatct

SEQ ID NO: 3 - DNA, 57 bp, synthetic construct
  source 1..57: mol_type = other DNA
tcttaccctatcagatttagccatgtgtagaccaaaggtctacacatgactaaatct

SEQ ID NO: 4 - DNA, 56 bp, synthetic construct
  source 1..56: mol_type = other DNA
tcttaccctatcagatttagccatgtgtagaccaaagtctacacatgactaaatct

SEQ ID NO: 5 - DNA, 56 bp, synthetic construct
  source 1..56: mol_type = other DNA
tcttaccctatcagatttagccatgtgtagaccaaagtctacacatggctaaatct

SEQ ID NO: 6 - DNA, 56 bp, synthetic construct
  source 1..56: mol_type = other DNA
tcttaccctatcagatttagccatgtgtagaccaaagtctacacatgactaaatgt

SEQ ID NO: 7 - DNA, 56 bp, synthetic construct
  source 1..56: mol_type = other DNA
tcttaccctatcagatttagccatgtgtagaccaaggtctacacatgactaaatct

SEQ ID NO: 8 - DNA, 56 bp, synthetic construct
  source 1..56: mol_type = other DNA
tcttaccctatcagatttagccatgtgtagaccagagtctacacatgactaaatct

SEQ ID NO: 9 - DNA, 56 bp, synthetic construct
  source 1..56: mol_type = other DNA
tcttaccctatcagatttagccatgtgtagaccgaagtctacacatgactaaatct

SEQ ID NO: 10 - DNA, 56 bp, synthetic construct
  source 1..56: mol_type = other DNA
tcttaccctatcagatttagccatgtgtagaccggggtctacacatgactaaatct

SEQ ID NO: 11 - DNA, 56 bp, synthetic construct
  source 1..56: mol_type = other DNA
tcttaccctatctgtactgcactcgaggcgtacaaatacgcctcgagagcagtaca

SEQ ID NO: 12 - DNA, 56 bp, synthetic construct
  source 1..56: mol_type = other DNA
tcttaccctatcagcacccagtccgccctgagcaaactcagggcggacagggtgct

SEQ ID NO: 13 - DNA, 56 bp, synthetic construct
  source 1..56: mol_type = other DNA
tcttaccctatcagatctagggatgtgtagaccaaagtctacacatcactagatct

SEQ ID NO: 14 - DNA, 56 bp, synthetic construct
  source 1..56: mol_type = other DNA
tcttaccctatcggatatacgcatctgtagaccaaagttcacagatgagtatatcc

SEQ ID NO: 15 - DNA, 44 bp, synthetic construct
  source 1..44: mol_type = other DNA
agactttggtctacacatggctaaatctttcatttttttttttt

SEQ ID NO: 16 - DNA, 28 bp, synthetic construct
  source 1..28: mol_type = other DNA
tttttttttttttgttgatagggtaaga

SEQ ID NO: 17 - DNA, 48 bp, synthetic construct
  source 1..48: mol_type = other DNA
agactttggtctacacatggctaaatctttcagacgtttttttttttt

SEQ ID NO: 18 - DNA, 32 bp, synthetic construct
  source 1..32: mol_type = other DNA
ttttttttttttcgtctgttgatagggtaaga

SEQ ID NO: 19 - DNA, 48 bp, synthetic construct
  source 1..48: mol_type = other DNA
agactttggtctacacatggctaaatctttcagacgacagtttttttt

SEQ ID NO: 20 - DNA, 32 bp, synthetic construct
  source 1..32: mol_type = other DNA
ttttttttctgtcgtctgttgatagggtaaga

SEQ ID NO: 21 - RNA, 41 nt, synthetic construct
  source 1..41: mol_type = other RNA
taatttctactaagtgtagatgtctacacatggctaaatct

SEQ ID NO: 22 - RNA, 41 nt, synthetic construct
  source 1..41: mol_type = other RNA
taatttctactaagtgtagatacatgacgtgagctccgcat

SEQ ID NO: 23 - RNA, 41 nt, synthetic construct
  source 1..41: mol_type = other RNA
taatttctactaagtgtagattcgtgggtcaggcgggactc

SEQ ID NO: 24 - RNA, 41 nt, synthetic construct
  source 1..41: mol_type = other RNA
taatttctactaagtgtagattctagatccctacacatctg

SEQ ID NO: 25 - RNA, 41 nt, synthetic construct
  source 1..41: mol_type = other RNA
taatttctactaagtgtagatcctatatgcgtagacatctg

SEQ ID NO: 26 - DNA, 40 bp, synthetic construct
  source 1..40: mol_type = other DNA
ccaatttggtctacacatggctaaatctgatagggtaaga

SEQ ID NO: 27 - DNA, 40 bp, synthetic construct
  source 1..40: mol_type = other DNA
accatttggtctacacatggctaaatctgatagggtaaga

SEQ ID NO: 28 - DNA, 40 bp, synthetic construct
  source 1..40: mol_type = other DNA
gacctttggtctacacatggctaaatctgatagggtaaga

SEQ ID NO: 29 - DNA, 40 bp, synthetic construct
  source 1..40: mol_type = other DNA
agactttggtctacacatggctaaatctgatagggtaaga

SEQ ID NO: 30 - DNA, 40 bp, synthetic construct
  source 1..40: mol_type = other DNA
agaccttggtctacacatggctaaatctgatagggtaaga

SEQ ID NO: 31 - DNA, 40 bp, synthetic construct
  source 1..40: mol_type = other DNA
agactctggtctacacatggctaaatctgatagggtaaga

SEQ ID NO: 32 - DNA, 40 bp, synthetic construct
  source 1..40: mol_type = other DNA
agacttcggtctacacatggctaaatctgatagggtaaga

SEQ ID NO: 33 - DNA, 40 bp, synthetic construct
  source 1..40: mol_type = other DNA
agaccccggtctacacatggctaaatctgatagggtaaga